European Patent Specification EP 4 157 876 B1, published September 4, 2024. Title: ANTI-PD-1 ANTIBODIES. Applicant: BOEHRINGER INGELHEIM INTERNATIONAL GMBH. The sequence listing filed with the application follows.

SEQUENCE LISTING (167 sequences)

SEQ ID NO: 1 - protein, 16 aa, Artificial Sequence
  source: /note="Description of Artificial Sequence: Synthetic peptide"
RSSKSLLHRNGITYLY

SEQ ID NO: 2 - protein, 7 aa, Artificial Sequence
  source: /note="Description of Artificial Sequence: Synthetic peptide"
EMSNLAS

SEQ ID NO: 3 - protein, 9 aa, Artificial Sequence
  source: /note="Description of Artificial Sequence: Synthetic peptide"
GQNLEFPLT

SEQ ID NO: 4 - protein, 11 aa, Artificial Sequence
  source: /note="Description of Artificial Sequence: Synthetic peptide"
KASQNVGTAVA

SEQ ID NO: 5 - protein, 7 aa, Artificial Sequence
  source: /note="Description of Artificial Sequence: Synthetic peptide"
SVSNRYT

SEQ ID NO: 6 - protein, 9 aa, Artificial Sequence
  source: /note="Description of Artificial Sequence: Synthetic peptide"
QQYSSYPFT

SEQ ID NO: 7 - protein, 11 aa, Artificial Sequence
  source: /note="Description of Artificial Sequence: Synthetic peptide"
HASQGINNNIG

SEQ ID NO: 8 - protein, 7 aa, Artificial Sequence
  source: /note="Description of Artificial Sequence: Synthetic peptide"
HKSNLED

SEQ ID NO: 9 - protein, 9 aa, Artificial Sequence
  source: /note="Description of Artificial Sequence: Synthetic peptide"
VQYAQFPYT

SEQ ID NO: 10 - protein, 16 aa, Artificial Sequence
  source: /note="Description of Artificial Sequence: Synthetic peptide"
RSSKSLLHRNGITYLY

SEQ ID NO: 11 - protein, 7 aa, Artificial Sequence
  source: /note="Description of Artificial Sequence: Synthetic peptide"
QMSNLAS

SEQ ID NO: 12 - protein, 9 aa, Artificial Sequence
  source: /note="Description of Artificial Sequence: Synthetic peptide"
AQNLELPLT

SEQ ID NO: 13 - protein, 17 aa, Artificial Sequence
  source: /note="Description of Artificial Sequence: Synthetic peptide"
KSSQSLLYSSNQKNYLA

SEQ ID NO: 14 - protein, 7 aa, Artificial Sequence
  source: /note="Description of Artificial Sequence: Synthetic peptide"
WASTRES

SEQ ID NO: 15 - protein, 9 aa, Artificial Sequence
  source: /note="Description of Artificial Sequence: Synthetic peptide"
HQYYSSPLT

SEQ ID NO: 16 - protein, 11 aa, Artificial Sequence
  source: /note="Description of Artificial Sequence: Synthetic peptide"
RASQEISGYLS

SEQ ID NO: 17 - protein, 7 aa, Artificial Sequence
  source: /note="Description of Artificial Sequence: Synthetic peptide"
AASTLDS

SEQ ID NO: 18 - protein, 9 aa, Artificial Sequence
  source: /note="Description of Artificial Sequence: Synthetic peptide"
LQYASYPLT

SEQ ID NO: 19 - protein, 10 aa, Artificial Sequence
  source: /note="Description of Artificial Sequence: Synthetic peptide"
SANSSVSFMH

SEQ ID NO: 20 - protein, 7 aa, Artificial Sequence
  source: /note="Description of Artificial Sequence: Synthetic peptide"
STSSLAS

SEQ ID NO: 21 - protein, 9 aa, Artificial Sequence
  source: /note="Description of Artificial Sequence: Synthetic peptide"
QQRSSYPLT

SEQ ID NO: 22 - protein, 11 aa, Artificial Sequence
  source: /note="Description of Artificial Sequence: Synthetic peptide"
KASQNVVTYVA

SEQ ID NO: 23 - protein, 7 aa, Artificial Sequence
  source: /note="Description of Artificial Sequence: Synthetic peptide"
SASYRYS

SEQ ID NO: 24 - protein, 9 aa, Artificial Sequence
  source: /note="Description of Artificial Sequence: Synthetic peptide"
QQYHSYPYT

SEQ ID NO: 25 - protein, 15 aa, Artificial Sequence
  source: /note="Description of Artificial Sequence: Synthetic peptide"
RASESVDIYGISFLH

SEQ ID NO: 26 - protein, 7 aa, Artificial Sequence
  source: /note="Description of Artificial Sequence: Synthetic peptide"
RASNLDS

SEQ ID NO: 27 - protein, 9 aa, Artificial Sequence
  source: /note="Description of Artificial Sequence: Synthetic peptide"
QQSNKDPLT

SEQ ID NO: 28 - protein, 17 aa, Artificial Sequence
  source: /note="Description of Artificial Sequence: Synthetic peptide"
KSSQSLLYSSNQKIYLA

SEQ ID NO: 29 - protein, 9 aa, Artificial Sequence
  source: /note="Description of Artificial Sequence: Synthetic peptide"
QQYYNSPLT

SEQ ID NO: 30 - protein, 12 aa, Artificial Sequence
  source: /note="Description of Artificial Sequence: Synthetic peptide"
SASSSISSDYLH

SEQ ID NO: 31 - protein, 7 aa, Artificial Sequence
  source: /note="Description of Artificial Sequence: Synthetic peptide"
RTSNLAS

SEQ ID NO: 32 - protein, 9 aa, Artificial Sequence
  source: /note="Description of Artificial Sequence: Synthetic peptide"
QQGTSLPRA

SEQ ID NO: 33 - protein, 17 aa, Artificial Sequence
  source: /note="Description of Artificial Sequence: Synthetic peptide"
KSSQSLLHSGNQKNYMT

SEQ ID NO: 34 - protein, 9 aa, Artificial Sequence
  source: /note="Description of Artificial Sequence: Synthetic peptide"
QNDYSYPLT

SEQ ID NO: 35 - protein, 7 aa, Artificial Sequence
  source: /note="Description of Artificial Sequence: Synthetic peptide"
VASTLDS

SEQ ID NO: 36 - protein, 9 aa, Artificial Sequence
  source: /note="Description of Artificial Sequence: Synthetic peptide"
LQYANYPYT

SEQ ID NO: 37 - protein, 11 aa, Artificial Sequence
  source: /note="Description of Artificial Sequence: Synthetic peptide"
SASQDIINYLN

SEQ ID NO: 38 - protein, 7 aa, Artificial Sequence
  source: /note="Description of Artificial Sequence: Synthetic peptide"
STSSLHS

SEQ ID NO: 39 - protein, 9 aa, Artificial Sequence
  source: /note="Description of Artificial Sequence: Synthetic peptide"
HQYSQLPYT

SEQ ID NO: 40 - protein, 11 aa, Artificial Sequence
  source: /note="Description of Artificial Sequence: Synthetic peptide"
SASQDIFNYLN

SEQ ID NO: 41 - protein, 7 aa, Artificial Sequence
  source: /note="Description of Artificial Sequence: Synthetic peptide"
YTSSLHS

SEQ ID NO: 42 - protein, 9 aa, Artificial Sequence
  source: /note="Description of Artificial Sequence: Synthetic peptide"
QQYSNLPYT

SEQ ID NO: 43 - protein, 10 aa, Artificial Sequence
  source: /note="Description of Artificial Sequence: Synthetic peptide"
GYTFTDYYVN

SEQ ID NO: 44 - protein, 17 aa, Artificial Sequence
  source: /note="Description of Artificial Sequence: Synthetic peptide"
DIHPNSGDTTYNQKFKD

SEQ ID NO: 45 - protein, 10 aa, Artificial Sequence
  source: /note="Description of Artificial Sequence: Synthetic peptide"
RRYDYDGFAY

SEQ ID NO: 46 - protein, 17 aa, Artificial Sequence
  source: /note="Description of Artificial Sequence: Synthetic peptide"
DIHPNNGGITYNQKFKG

SEQ ID NO: 47 - protein, 10 aa, Artificial Sequence
  source: /note="Description of Artificial Sequence: Synthetic peptide"
GFTFSDYGMH

SEQ ID NO: 48 - protein, 17 aa, Artificial Sequence
  source: /note="Description of Artificial Sequence: Synthetic peptide"
YINSDSNTIYYADTVKG

SEQ ID NO: 49 - protein, 6 aa, Artificial Sequence
  source: /note="Description of Artificial Sequence: Synthetic peptide"
LVAPDY

SEQ ID NO: 50 - protein, 10 aa, Artificial Sequence
  source: /note="Description of Artificial Sequence: Synthetic peptide"
GHTFTSNWIH

SEQ ID NO: 51 - protein, 17 aa, Artificial Sequence
  source: /note="Description of Artificial Sequence: Synthetic peptide"
EIDPSDSYTYYNQKFKG

SEQ ID NO: 52 - protein, 9 aa, Artificial Sequence
  source: /note="Description of Artificial Sequence: Synthetic peptide"
PGRNSNFAY

SEQ ID NO: 53 - protein, 12 aa, Artificial Sequence
  source: /note="Description of Artificial Sequence: Synthetic peptide"
GFSLSTSGMGVT

SEQ ID NO: 54 - protein, 16 aa, Artificial Sequence
  source: /note="Description of Artificial Sequence: Synthetic peptide"
HIFWDGDKRYNPSLKS

SEQ ID NO: 55 - protein, 12 aa, Artificial Sequence
  source: /note="Description of Artificial Sequence: Synthetic peptide"
YYYFDYGYAIDY

SEQ ID NO: 56 - protein, 10 aa, Artificial Sequence
  source: /note="Description of Artificial Sequence: Synthetic peptide"
GYTFTSYVIH

SEQ ID NO: 57 - protein, 17 aa, Artificial Sequence
  source: /note="Description of Artificial Sequence: Synthetic peptide"
YIDPSNDDTKYNEKFKG

SEQ ID NO: 58 - protein, 12 aa, Artificial Sequence
  source: /note="Description of Artificial Sequence: Synthetic peptide"
EAYYGGLYGMDY

SEQ ID NO: 59 - protein, 10 aa, Artificial Sequence
  source: /note="Description of Artificial Sequence: Synthetic peptide"
GYTFIDYTIH

SEQ ID NO: 60 - protein, 18 aa, Artificial Sequence
  source: /note="Description of Artificial Sequence: Synthetic peptide"
WIFPGSTNDTKYNDKFKG

SEQ ID NO: 61 - protein, 7 aa, Artificial Sequence
  source: /note="Description of Artificial Sequence: Synthetic peptide"
YRTDFDY

SEQ ID NO: 62 - protein, 10 aa, Artificial Sequence
  source: /note="Description of Artificial Sequence: Synthetic peptide"
GYSFTSYWMH

SEQ ID NO: 63 - protein, 17 aa, Artificial Sequence
  source: /note="Description of Artificial Sequence: Synthetic peptide"
DIDPSNSYAYHSQKFKG

SEQ ID NO: 64 - protein, 11 aa, Artificial Sequence
  source: /note="Description of Artificial Sequence: Synthetic peptide"
ADGTSHWYFDV

SEQ ID NO: 65 - protein, 10 aa, Artificial Sequence
  source: /note="Description of Artificial Sequence: Synthetic peptide"
GYTFTDYYLN

SEQ ID NO: 66 - protein, 17 aa, Artificial Sequence
  source: /note="Description of Artificial Sequence: Synthetic peptide"
WIYPGSSDTKHNENFKG

SEQ ID NO: 67 - protein, 8 aa, Artificial Sequence
  source: /note="Description of Artificial Sequence: Synthetic peptide"
YSNFFFDY

SEQ ID NO: 68 - protein, 12 aa, Artificial Sequence
  source: /note="Description of Artificial Sequence: Synthetic peptide"
GFSLSTSGMGVS

SEQ ID NO: 69 - protein, 16 aa, Artificial Sequence
  source: /note="Description of Artificial Sequence: Synthetic peptide"
HIYWDDDKRYNPSLKS

SEQ ID NO: 70 - protein, 11 aa, Artificial Sequence
  source: /note="Description of Artificial Sequence: Synthetic peptide"
SSQGLYSSYDY

SEQ ID NO: 71 - protein, 10 aa, Artificial Sequence
  source: /note="Description of Artificial Sequence: Synthetic peptide"
GYTFTSYVMH

SEQ ID NO: 72 - protein, 17 aa, Artificial Sequence
  source: /note="Description of Artificial Sequence: Synthetic peptide"
YIDPDNDGTKYNEKFKG

SEQ ID NO: 73 - protein, 10 aa, Artificial Sequence
  source: /note="Description of Artificial Sequence: Synthetic peptide"
GFTFSDYYMS

SEQ ID NO: 74 - protein, 17 aa, Artificial Sequence
  source: /note="Description of Artificial Sequence: Synthetic peptide"
YISSGGGSSYYPDSVKG

SEQ ID NO: 75 - protein, 9 aa, Artificial Sequence
  source: /note="Description of Artificial Sequence: Synthetic peptide"
LPHYFAMDC

SEQ ID NO: 76 - protein, 17 aa, Artificial Sequence
  source: /note="Description of Artificial Sequence: Synthetic peptide"
YISSGGGSKYYPDLVKG

SEQ ID NO: 77 - protein, 9 aa, Artificial Sequence
  source: /note="Description of Artificial Sequence: Synthetic peptide"
LPHYFAMDY

SEQ ID NO: 78 - protein, 17 aa, Artificial Sequence
  source: /note="Description of Artificial Sequence: Synthetic peptide"
YISSGGGSSYYPDAVKG

SEQ ID NO: 79 - protein, 17 aa, Artificial Sequence
  source: /note="Description of Artificial Sequence: Synthetic peptide"
YISSGGGSSYYPDLVKG

SEQ ID NO: 80 - protein, 10 aa, Artificial Sequence
  source: /note="Description of Artificial Sequence: Synthetic peptide"
GFTFSDYYMA

SEQ ID NO: 81 - protein, 17 aa, Artificial Sequence
  source: /note="Description of Artificial Sequence: Synthetic peptide"
NINYDGFNTYYLDSLKS

SEQ ID NO: 82 - protein, 10 aa, Artificial Sequence
  source: /note="Description of Artificial Sequence: Synthetic peptide"
GGYWSLYFDY

SEQ ID NO: 83 - protein, 10 aa, Artificial Sequence
  source: /note="Description of Artificial Sequence: Synthetic peptide"
GYTFTDYYIN

SEQ ID NO: 84 - protein, 17 aa, Artificial Sequence
  source: /note="Description of Artificial Sequence: Synthetic peptide"
WIYPGGGHTKYNEKFKG

SEQ ID NO: 85 - protein, 8 aa, Artificial Sequence
  source: /note="Description of Artificial Sequence: Synthetic peptide"
YSNYYFDF

SEQ ID NO: 86 - protein, 10 aa, Artificial Sequence
  source: /note="Description of Artificial Sequence: Synthetic peptide"
GYTFTSYYIQ

SEQ ID NO: 87 - protein, 17 aa, Artificial Sequence
  source: /note="Description of Artificial Sequence: Synthetic peptide"
WIYPGDGTTNYNENFKG

SEQ ID NO: 88 - protein, 8 aa, Artificial Sequence
  source: /note="Description of Artificial Sequence: Synthetic peptide"
YGLVPFDY

SEQ ID NO: 89 - protein, 10 aa, Artificial Sequence
  source: /note="Description of Artificial Sequence: Synthetic peptide"
GNTFNSNYIQ

SEQ ID NO: 90 - protein, 17 aa, Artificial Sequence
  source: /note="Description of Artificial Sequence: Synthetic peptide"
WIYPGDGSTNYSEKFKG

SEQ ID NO: 91 - protein, 8 aa, Artificial Sequence
  source: /note="Description of Artificial Sequence: Synthetic peptide"
YGPVPFDY

SEQ ID NO: 92 - protein, 112 aa, Artificial Sequence
  source: /note="Description of Artificial Sequence: Synthetic polypeptide"
EIVMTQAAFSNPVTLGTSASISCRSSKSLLHRNGITYLYWYLQKPGQSPQLLIYEMSNLASGVPDRFSSSGSGTDFTLRISRVEAEDVGVYYCGQNLEFPLTFGAGTKLELK

SEQ ID NO: 93 - protein, 112 aa, Artificial Sequence
  source: /note="Description of Artificial Sequence: Synthetic polypeptide"
EIVMTQAAFSNPVTLGTSASISCRSSKSLLHRNGITYLYWYLQKPGQSPQLLIYEMSNLASGVPDRFSGSGSGTDFTLRISRVEAEDVGVYYCGQNLEFPLTFGAGTKLELK

SEQ ID NO: 94 - protein, 107 aa, Artificial Sequence
  source: /note="Description of Artificial Sequence: Synthetic polypeptide"
DIVMTQSQKFMSTTVGDRVSITCKASQNVGTAVAWYQQKPGQSPKLLIYSVSNRYTGVPDRFTGSGSGTDFTLTISNMQSEDLADYFCQQYSSYPFTFGAGTKLELK

SEQ ID NO: 95 - protein, 107 aa, Artificial Sequence
  source: /note="Description of Artificial Sequence: Synthetic polypeptide"
DILMTQSPSSMSVSLGDTVSITCHASQGINNNIGWLQQKPGKSFKGLIYHKSNLEDGVPSRFSGSGSGADYSLTISSLESEDFADYYCVQYAQFPYTFGGGTKLEIK

SEQ ID NO: 96 - protein, 112 aa, Artificial Sequence
  source: /note="Description of Artificial Sequence: Synthetic polypeptide"
DIVMTQAAFYNPVTLGTSASISCRSSKSLLHRNGITYLYWYLQKPGQSPQLLIYQMSNLASGVPDRFSSSGSGADFTLRISRVEAEDVGVYYCAQNLELPLTFGAGTKLELK

SEQ ID NO: 97 - protein, 113 aa, Artificial Sequence
  source: /note="Description of Artificial Sequence: Synthetic polypeptide"
DIVMSQSPSSLAVSVGEKVTMTCKSSQSLLYSSNQKNYLAWYQQKPGQSPKLLIYWASTRESGVPDRFTGSGSGTDFTLTISSVKAEDLAVYYCHQYYSSPLTFGAGTKLELK

SEQ ID NO: 98 - protein, 107 aa, Artificial Sequence
  source: /note="Description of Artificial Sequence: Synthetic polypeptide"
DIQMTQSPSSLSASLGERVSLTCRASQEISGYLSWLQQKPDGTIKRLIYAASTLDSGVPKRFSGSRSGSDYSLTISSLESEDFADYYCLQYASYPLTFGAGTKLELK

SEQ ID NO: 99 - protein, 106 aa, Artificial Sequence
  source: /note="Description of Artificial Sequence: Synthetic polypeptide"
QIVLTQSPGIMSASPGEKVTITCSANSSVSFMHWFQQKPGTSPKIWIYSTSSLASGVPARFSGSGSGTSYSLTISRMEAEDAATYYCQQRSSYPLTFGAGTKLELK

SEQ ID NO: 100 - protein, 107 aa, Artificial Sequence
  source: /note="Description of Artificial Sequence: Synthetic polypeptide"
DIVMTQSQKFLSTSVGDRVRVTCKASQNVVTYVAWYQQKPGQSPKSLIYSASYRYSGVPDRFTGSGSGTYFTLTINNVQFEDLAEYFCQQYHSYPYTFGGGTKLEIK

SEQ ID NO: 101 - protein, 111 aa, Artificial Sequence
  source: /note="Description of Artificial Sequence: Synthetic polypeptide"
DIVLTQSPASLAVSLGQRATISCRASESVDIYGISFLHWYQQKPGQPPKHLIYRASNLDSGIPARFSGSGSRTDFTLTINPVETDDVATYYCQQSNKDPLTFGAGTKLELK

SEQ ID NO: 102 - protein, 113 aa, Artificial Sequence
  source: /note="Description of Artificial Sequence: Synthetic polypeptide"
DIVMSQSPSSLTVSVGEKVTMSCKSSQSLLYSSNQKIYLAWFQQKPGQSPKLLIYWASTRESGVPDRFTGSGSGTDFTLTISSVKAEDLAVYYCQQYYNSPLTFGAGTKLELK

SEQ ID NO: 103 - protein, 108 aa, Artificial Sequence
  source: /note="Description of Artificial Sequence: Synthetic polypeptide"
EIVLTQSPTTMAASPGEKITITCSASSSISSDYLHWYQQKPGFSPELLIYRTSNLASGVPARFSGSGSGTSYSLTIGSMEAEDVATYYCQQGTSLPRAFGGGTKLEIK

SEQ ID NO: 104 - protein, 113 aa, Artificial Sequence
  source: /note="Description of Artificial Sequence: Synthetic polypeptide"
DIVMTQSPSSLTVTAGEKVTMSCKSSQSLLHSGNQKNYMTWYQQKPGQPPKLLIYWASTRESGVPDRFTGSGSGTDFTLTISSVQAEDLAVYYCQNDYSYPLTFGAGTKLELK

SEQ ID NO: 105 - protein, 107 aa, Artificial Sequence
  source: /note="Description of Artificial Sequence: Synthetic polypeptide"
DIQMTQSPSSLSASPGERVSLTCRASQEISGYLSWLQQKPDGTIKRLIYVASTLDSGVPKRFSGSRSGSDYSLTISSLESEDFADYYCLQYANYPYTFGGGTKLEIK

SEQ ID NO: 106 - protein, 107 aa, Artificial Sequence
  source: /note="Description of Artificial Sequence: Synthetic polypeptide"
DIQMTQTTSSLSASLGDRVTISCSASQDIINYLNWYQQKPDGTVKLLIYSTSSLHSGVSLRFSGSGSGTDYSLTISNLEPEDVATYYCHQYSQLPYTFGGGTKLEIK

SEQ ID NO: 107 - protein, 107 aa, Artificial Sequence
  source: /note="Description of Artificial Sequence: Synthetic polypeptide"
DIQMTQTTSSLSASLGDRVTISCSASQDIFNYLNWYQQKPDGTVKLLIYYTSSLHSGVPSRFSGSGSGTDFSLTISNLEPEDIATYYCQQYSNLPYTFGGGTKLEIK

SEQ ID NO: 108 - protein, 119 aa, Artificial Sequence
  source: /note="Description of Artificial Sequence: Synthetic polypeptide"
EVQLQQSGPELVKPGSSVKISCKASGYTFTDYYVNWVKQSHGKSLEWFGDIHPNSGDTTYNQKFKDKATLTVDKSSSTAYMELRSLTSEDSAVYYCARRRYDYDGFAYWGQGTLVTVSA

SEQ ID NO: 109 - protein, 119 aa, Artificial Sequence
  source: /note="Description of Artificial Sequence: Synthetic polypeptide"
EVQLQQSGPELVKPGASVKISCKASGYTFTDYYVNWVKQSHGKSLEWFGDIHPNNGGITYNQKFKGKASLTVDKSSSTAYMELRSLTSEDSAVYYCARRRYDYDGFAYWGQGTLVTVSA

SEQ ID NO: 110 - protein, 115 aa, Artificial Sequence
  source: /note="Description of Artificial Sequence: Synthetic polypeptide"
EVQLVESGGGLVKPGGSLKLSCAASGFTFSDYGMHWVRQTPEKGLEWIAYINSDSNTIYYADTVKGRFTISRDNARKTLYLQMTSLRSEDTAMYYCSPLVAPDYWGQGTTLTVSS

SEQ ID NO: 111 - protein, 118 aa, Artificial Sequence
  source: /note="Description of Artificial Sequence: Synthetic polypeptide"
QVQLQQPGAELVKPGASVKLSCKASGHTFTSNWIHWVKQRPGQGLEWIGEIDPSDSYTYYNQKFKGKATLTVDKSSSTAYMQLSSLTSEDSAVYSCACPGRNSNFAYWGQGTTLTVSS

SEQ ID NO: 112 - protein, 122 aa, Artificial Sequence
  source: /note="Description of Artificial Sequence: Synthetic polypeptide"
QVTLKESGPGILQPSQTLSLTCSFSGFSLSTSGMGVTWIRKPSGQGLEWLAHIFWDGDKRYNPSLKSRLTISKDSSSNQVFLMITGVGTADAATYYCARYYYFDYGYAIDYWGQGTSVTVSS

SEQ ID NO: 113 - protein, 121 aa, Artificial Sequence
  source: /note="Description of Artificial Sequence: Synthetic polypeptide"
EVQLQQSGPELVKPGASVKMSCKASGYTFTSYVIHWVKQKPGQGLEWIGYIDPSNDDTKYNEKFKGKATLTSDKSSSTAYMELSSLTSEDSAVYYCAREAYYGGLYGMDYWGQGTSVTVSS

SEQ ID NO: 114 - protein, 117 aa, Artificial Sequence
  source: /note="Description of Artificial Sequence: Synthetic polypeptide"
QVQLQQSGPELVKPGASVKLSCKASGYTFIDYTIHWVKQSPGQGLEWIGWIFPGSTNDTKYNDKFKGKATMTADKSSSTAYMQLSSLTSEDSAVYFCARYRTDFDYWGQGTTLTVSS

SEQ ID NO: 115 - protein, 120 aa, Artificial Sequence
  source: /note="Description of Artificial Sequence: Synthetic polypeptide"
QVQLQQPGAELVKPGASVKLSCKASGYSFTSYWMHWVRQRPGQGLEWIGDIDPSNSYAYHSQKFKGKATLTVDKSSSTAYMQLSSLTSEDSAVYFCARADGTSHWYFDVWGAGTAVTVSS

SEQ ID NO: 116 - protein, 117 aa, Artificial Sequence
  source: /note="Description of Artificial Sequence: Synthetic polypeptide"
QIQLQQSGPELVKPGASVKISCKASGYTFTDYYLNWVKQRPGHGLEWIGWIYPGSSDTKHNENFKGKATLTVDTYSSTAYMQLGSLTSEDSAVYFCTRYSNFFFDYWGQGTTLTVSS

SEQ ID NO: 117 - protein, 121 aa, Artificial Sequence
  source: /note="Description of Artificial Sequence: Synthetic polypeptide"
QVTLKESGPGILQPSQTLSLTCSFSGFSLSTSGMGVSWIRQPSGKGLEWLTHIYWDDDKRYNPSLKSRLTISKDTSRNQVFLEITSVDTADTATYFCARSSQGLYSSYDYWGQGTTLTVSS

SEQ ID NO: 118 - protein, 121 aa, Artificial Sequence
  source: /note="Description of Artificial Sequence: Synthetic polypeptide"
EVQLQQSGPELVKPGASVKMSCKASGYTFTSYVMHWVRQKPGQGLEWIGYIDPDNDGTKYNEKFKGKATLTSDKSSSTAYMELSSLTSEDSAVYYCAREAYYGGLYGMDYWGQGSSVTVSS

SEQ ID NO: 119 - protein, 118 aa, Artificial Sequence
  source: /note="Description of Artificial Sequence: Synthetic polypeptide"
EVQLVESGGGLVQPGGSLKLSCAASGFTFSDYYMSWVRQTPEKRLEWVAYISSGGGSSYYPDSVKGRFTISRDNTKNTLYLQMSSLKSEDTAVYYCARLPHYFAMDCWGQGTSVTVSS

SEQ ID NO: 120 - protein, 119 aa, Artificial Sequence
  source: /note="Description of Artificial Sequence: Synthetic polypeptide"
EVKLVESEGGLVQPGSSMKLSCTASGFTFSDYYMAWVRQVPEKGLEWVANINYDGFNTYYLDSLKSRFIISRDNAKNILYLQMSSLKSEDTATYYCARGGYWSLYFDYWGQGTTLTVSS

SEQ ID NO: 121 - protein, 117 aa, Artificial Sequence
  source: /note="Description of Artificial Sequence: Synthetic polypeptide"
QIQLQQSGPEVVKPGASVKISCKASGYTFTDYYINWVKQRPGQGLEWIGWIYPGGGHTKYNEKFKGEATLTVDTSSRTAYMQLSSLTSEDSAVYFCARYSNYYFDFWGHGTTLTVSS

SEQ ID NO: 122 - protein, 117 aa, Artificial Sequence
  source: /note="Description of Artificial Sequence: Synthetic polypeptide"
QIQLQQSGPELVKPGASVKISCKASGYTFTSYYIQWVKQRPGQGLEWIGWIYPGDGTTNYNENFKGKTTLTADKSSSTVYMLLSSLTSEDSAVYFCARYGLVPFDYWGQGTTLTVSS

SEQ ID NO: 123 - protein, 117 aa, Artificial Sequence
  source: /note="Description of Artificial Sequence: Synthetic polypeptide"
QIQLQQSGPELVKTGASVKISCKASGNTFNSNYIQWVKQRPGQGLEWIGWIYPGDGSTNYSEKFKGKTTLTADKSSSTAYMLVSSLTSEDSAVYFCARYGPVPFDYWGQGTTLSVSS

SEQ ID NO: 124 - DNA, 324 bp, Artificial Sequence
  source: /note="Description of Artificial Sequence: Synthetic polynucleotide"
gatatccagatgacgcagagcccaagcagcctgagcgcgtccgtgggcgaccgcgtgacgatcacctgtagcgcgtcccagagcatcagcagcgactatctgcattggtatcagcagaaaccaggtaaagcccctaaactgctgatctaccggacctccaatctggcaagcggcgtgcctagccgtttcagcggtagcggctccggtaccgacttcacctttactatctccagcctgcagcctgaagacatcgcgacgtattattgtcagcagggtactagcctgcctcgcgccttcggccaggggaccaaactggaaatcaaa

SEQ ID NO: 125 - protein, 108 aa, Artificial Sequence
  source: /note="Description of Artificial Sequence: Synthetic polypeptide"
DIQMTQSPSSLSASVGDRVTITCSASQSISSDYLHWYQQKPGKAPKLLIYRTSNLASGVPSRFSGSGSGTDFTFTISSLQPEDIATYYCQQGTSLPRAFGQGTKLEIK

SEQ ID NO: 126 - DNA, 324 bp, Artificial Sequence
  source: /note="Description of Artificial Sequence: Synthetic polynucleotide"
gatatccagatgacgcagagcccaagcagcctgagcgcgtccgtgggcgaccgcgtgacgatcacctgtcaggcgtcccagagcatcagcagcgactatctgcattggtatcagcagaaaccaggtaaagcccctaaactgctgatctaccggacctccaatctggaaaccggcgtgcctagccgtttcagcggtagcggctccggtaccgacttcacctttactatctccagcctgcagcctgaagacatcgcgacgtattattgtcagcagggtactagcctgcctcgcgccttcggccaggggaccaaactggaaatcaaa

SEQ ID NO: 127 - protein, 108 aa, Artificial Sequence
  source: /note="Description of Artificial Sequence: Synthetic polypeptide"
DIQMTQSPSSLSASVGDRVTITCQASQSISSDYLHWYQQKPGKAPKLLIYRTSNLETGVPSRFSGSGSGTDFTFTISSLQPEDIATYYCQQGTSLPRAFGQGTKLEIK

SEQ ID NO: 128 - DNA, 324 bp, Artificial Sequence
  source: /note="Description of Artificial Sequence: Synthetic polynucleotide"
gatatccagatgacgcagagcccaagcagcctgagcgcgtccgtgggcgaccgcgtgacgatcacctgtcaggcgtcccagagcatcagcagcgactatctgcattggtatcagcagaaaccaggtaaagcccctaaactgctgatctaccggacctccaatctggaaagcggcgtgcctagccgtttcagcggtagcggctccggtaccgacttcacctttactatctccagcctgcagcctgaagacatcgcgacgtattattgtcagcagggtactagcctgcctcgcgccttcggccaggggaccaaactggaaatcaaa

SEQ ID NO: 129 - protein, 108 aa, Artificial Sequence
  source: /note="Description of Artificial Sequence: Synthetic polypeptide"
DIQMTQSPSSLSASVGDRVTITCQASQSISSDYLHWYQQKPGKAPKLLIYRTSNLESGVPSRFSGSGSGTDFTFTISSLQPEDIATYYCQQGTSLPRAFGQGTKLEIK

SEQ ID NO: 130 - DNA, 354 bp, Artificial Sequence
  source: /note="Description of Artificial Sequence: Synthetic polynucleotide"
gaagtgcagctggtggaaagcggtggtggcctggtgcagccaggcggctccctgcgcctgagctgcgccgcaagcggtttcacctttagcgactactatatgtcctgggtgcgtcaggcgccaggtaaaggtctggaatgggtgtcatacatcagctccgggggcggtagcaagtactatccggacctggtgaaagggcgctttactatctcccgggataatgcaaaaaatagcctgtacctgcagatgagcagcctgcgggcggaagataccgccgtgtattactgtgcgcgtctgccgcattatttcgccatggattactggggccaggggaccctggtgaccgtgagcagc

SEQ ID NO: 131 - protein, 118 aa, Artificial Sequence
  source: /note="Description of Artificial Sequence: Synthetic polypeptide"
EVQLVESGGGLVQPGGSLRLSCAASGFTFSDYYMSWVRQAPGKGLEWVSYISSGGGSKYYPDLVKGRFTISRDNAKNSLYLQMSSLRAEDTAVYYCARLPHYFAMDYWGQGTLVTVSS

SEQ ID NO: 132 - DNA, 354 bp, Artificial Sequence
  source: /note="Description of Artificial Sequence: Synthetic polynucleotide"
gaagtgcagctggtggaaagcggtggtggcctggtgcagccaggcggctccctgcgcctgagctgcgccgcaagcggtttcacctttagcgactactatatgtcctgggtgcgtcaggcgccaggtaaaggtctggaatgggtggcatacatcagctccgggggcggtagcagctactatccggacctggtgaaagggcgctttactatctcccgggataatgcaaaaaatagcctgtacctgcagatgcagagcctgcgggcggaagataccgccgtgtattactgtgcgcgtctgccgcattatttcgccatggattactggggccaggggaccctggtgaccgtgagcagc

SEQ ID NO: 133 - protein, 118 aa, Artificial Sequence
  source: /note="Description of Artificial Sequence: Synthetic polypeptide"
EVQLVESGGGLVQPGGSLRLSCAASGFTFSDYYMSWVRQAPGKGLEWVAYISSGGGSSYYPDLVKGRFTISRDNAKNSLYLQMQSLRAEDTAVYYCARLPHYFAMDYWGQGTLVTVSS

SEQ ID NO: 134 - DNA, 354 bp, Artificial Sequence
  source: /note="Description of Artificial Sequence: Synthetic polynucleotide"
gaagtgcagctggtggaaagcggtggtggcctggtgcagccaggcggctccctgcgcctgagctgcgccgcaagcggtttcacctttagcgactactatatgtcctgggtgcgtcaggcgccaggtaaaggtctggaatgggtggcatacatcagctccgggggcggtagcagctactatccggacgctgtgaaagggcgctttactatctcccgggataatgcaaaacagagcctgtacctgcagatgcagagcctgcgggcggaagataccgccgtgtattactgtgcgcgtctgccgcattatttcgccatggattactggggccaggggaccctggtgaccgtgagcagc

SEQ ID NO: 135 - protein, 118 aa, Artificial Sequence
  source: /note="Description of Artificial Sequence: Synthetic polypeptide"
EVQLVESGGGLVQPGGSLRLSCAASGFTFSDYYMSWVRQAPGKGLEWVAYISSGGGSSYYPDAVKGRFTISRDNAKQSLYLQMQSLRAEDTAVYYCARLPHYFAMDYWGQGTLVTVSS

SEQ ID NO: 136 - DNA, 354 bp, Artificial Sequence
  source: /note="Description of Artificial Sequence: Synthetic polynucleotide"
gaagtgcagctggtggaaagcggtggtggcctggtgcagccaggcggctccctgcgcctgagctgcgccgcaagcggtttcacctttagcgactactatatgtcctgggtgcgtcaggcgccaggtaaaggtctggaatgggtggcctacatcagctccgggggcggtagcagctactatccggacctggtgaaagggcgctttactatctcccgggataatgcaaaacagagcctgtacctgcagatgaacagcctgcgggcggaagataccgccgtgtattactgtgcgcgtctgccgcattatttcgccatggattactggggccaggggaccctggtgaccgtgagcagc

SEQ ID NO: 137 - protein, 118 aa, Artificial Sequence
  source: /note="Description of Artificial Sequence: Synthetic polypeptide"
EVQLVESGGGLVQPGGSLRLSCAASGFTFSDYYMSWVRQAPGKGLEWVAYISSGGGSSYYPDLVKGRFTISRDNAKQSLYLQMNSLRAEDTAVYYCARLPHYFAMDYWGQGTLVTVSS

SEQ ID NO: 138 - DNA, 354 bp, Artificial Sequence
  source: /note="Description of Artificial Sequence: Synthetic polynucleotide"
gaagtgcagctggtggaaagcggtggtggcctggtgcagccaggcggctccctgcgcctgagctgcgccgcaagcggtttcacctttagcgactactatatgtcctgggtgcgtcaggcgccaggtaaaggtctggaatgggtggcctacatcagctccgggggcggtagcagctactatccggacctggtgaaagggcgctttactatctcccgggataatgcaaaacagagcctgtacctgcagatgcagagcctgcgggcggaagataccgccgtgtattactgtgcgcgtctgccgcattatttcgccatggattactggggccaggggaccctggtgaccgtgagcagc

SEQ ID NO: 139 - protein, 118 aa, Artificial Sequence
  source: /note="Description of Artificial Sequence: Synthetic polypeptide"
EVQLVESGGGLVQPGGSLRLSCAASGFTFSDYYMSWVRQAPGKGLEWVAYISSGGGSSYYPDLVKGRFTISRDNAKQSLYLQMQSLRAEDTAVYYCARLPHYFAMDYWGQGTLVTVSS

SEQ ID NO: 140 - DNA, 645 bp, Artificial Sequence
  source: /note="Description of Artificial Sequence: Synthetic polynucleotide"
gatatccagatgacgcagagcccaagcagcctgagcgcgtccgtgggcgaccgcgtgacgatcacctgtagcgcgtcccagagcatcagcagcgactatctgcattggtatcagcagaaaccaggtaaagcccctaaactgctgatctaccggacctccaatctggcaagcggcgtgcctagccgtttcagcggtagcggctccggtaccgacttcacctttactatctccagcctgcagcctgaagacatcgcgacgtattattgtcagcagggtactagcctgcctcgcgccttcggccaggggaccaaactggaaatcaaacgtactgtggctgcaccatctgtcttcatcttcccgccatctgatgagcaattgaaatctggaactgcctctgttgtgtgcctgctgaataacttctatcccagagaggccaaagtacagtggaaggtggataacgccctccaatcgggtaactcccaggagagtgtcacagagcaggacagcaaggacagcacctacagcctcagcagcaccctgacgctgagcaaagcagactacgagaaacacaaagtctacgcctgcgaagtcacccatcagggcctgagctcgcccgtcacaaagagcttcaacaggggagagtgt

SEQ ID NO: 141 - protein, 215 aa, Artificial Sequence
  source: /note="Description of Artificial Sequence: Synthetic polypeptide"
DIQMTQSPSSLSASVGDRVTITCSASQSISSDYLHWYQQKPGKAPKLLIYRTSNLASGVPSRFSGSGSGTDFTFTISSLQPEDIATYYCQQGTSLPRAFGQGTKLEIKRTVAAPSVFIFPPSDEQLKSGTASVVCLLNNFYPREAKVQWKVDNALQSGNSQESVTEQDSKDSTYSLSSTLTLSKADYEKHKVYACEVTHQGLSSPVTKSFNRGEC

SEQ ID NO: 142 - DNA, 1332 bp, Artificial Sequence
  source: /note="Description of Artificial Sequence: Synthetic polynucleotide"
gaagtgcagctggtggaaagcggtggtggcctggtgcagccaggcggctccctgcgcctgagctgcgccgcaagcggtttcacctttagcgactactatatgtcctgggtgcgtcaggcgccaggtaaaggtctggaatgggtgtcatacatcagctccgggggcggtagcaagtactatccggacctggtgaaagggcgctttactatctcccgggataatgcaaaaaatagcctgtacctgcagatgagcagcctgcgggcggaagataccgccgtgtattactgtgcgcgtctgccgcattatttcgccatggattactggggccaggggaccctggtgaccgtgagcagcgcctccacaaagggcccttccgtgttccccctggccccttgctcccggtccacctccgagtctaccgccgctctgggctgcctggtcaaggactacttccccgagcccgtgaccgtgtcctggaactctggcgccctgacctccggcgtgcacaccttccctgctgtgctgcagtcctccggcctgtactccctgtcctccgtcgtgaccgtgccctcctctagcctgggcaccaagacctacacctgtaacgtggaccacaagccctccaacaccaaggtggacaagcgggtggaatctaagtacggccctccctgccccccctgccctgcccctgaatttctgggcggaccctccgtgttcctgttccccccaaagcccaaggacaccctgatgatctcccggacccccgaagtgacctgcgtggtggtggacgtgtcccaggaagatcccgaggtccagtttaattggtacgtggacggcgtggaagtgcacaacgccaagaccaagcccagagaggaacagttcaactccacctaccgggtggtgtccgtgctgaccgtgctgcaccaggactggctgaacggcaaagagtacaagtgcaaggtgtccaacaagggcctgccctccagcatcgaaaagaccatctccaaggccaagggccagccccgcgagccccaggtgtacaccctgcctccaagccaggaagagatgaccaagaaccaggtgtccctgacctgtctggtcaagggcttctacccctccgatatcgccgtggaatgggagtccaacggccagcccgagaacaactacaagaccaccccccctgtgctggactccgacggctccttcttcctgtactctcggctgaccgtggacaagtcccggtggcaggaaggcaacgtcttctcctgctccgtgatgcacgaggccctgcacaaccactacacccagaagtccctgtccctgagcctgggc

SEQ ID NO: 143 - protein, 444 aa, Artificial Sequence
  source: /note="Description of Artificial Sequence: Synthetic polypeptide"
EVQLVESGGGLVQPGGSLRLSCAASGFTFSDYYMSWVRQAPGKGLEWVSYISSGGGSKYYPDLVKGRFTISRDNAKNSLYLQMSSLRAEDTAVYYCARLPHYFAMDYWGQGTLVTVSSASTKGPSVFPLAPCSRSTSESTAALGCLVKDYFPEPVTVSWNSGALTSGVHTFPAVLQSSGLYSLSSVVTVPSSSLGTKTYTCNVDHKPSNTKVDKRVESKYGPPCPPCPAPEFLGGPSVFLFPPKPKDTLMISRTPEVTCVVVDVSQEDPEVQFNWYVDGVEVHNAKTKPREEQFNSTYRVVSVLTVLHQDWLNGKEYKCKVSNKGLPSSIEKTISKAKGQPREPQVYTLPPSQEEMTKNQVSLTCLVKGFYPSDIAVEWESNGQPENNYKTTPPVLDSDGSFFLYSRLTVDKSRWQEGNVFSCSVMHEALHNHYTQKSLSLSLG

SEQ ID NO: 144 - DNA, 645 bp, Artificial Sequence
  source: /note="Description of Artificial Sequence: Synthetic polynucleotide"
gacatccagatgacccagagcccaagcagcctgagcgccagcgtgggcgaccgcgtgaccatcacctgccaggccagccagagcatcagcagcgactacctgcactggtaccagcagaagccaggcaaggccccaaagctgctgatctaccgcaccagcaacctggagaccggcgtgccaagccgcttcagcggcagcggcagcggcaccgacttcaccttcaccatcagcagcctgcagccagaggacatcgccacctactactgccagcagggcaccagcctgccacgcgccttcggccagggcaccaagctggagatcaagcgtactgtggctgcaccatctgtcttcatcttcccgccatctgatgagcaattgaaatctggaactgcctctgttgtgtgcctgctgaataacttctatcccagagaggccaaagtacagtggaaggtggataacgccctccaatcgggtaactcccaggagagtgtcacagagcaggacagcaaggacagcacctacagcctcagcagcaccctgacgctgagcaaagcagactacgagaaacacaaagtctacgcctgcgaagtcacccatcagggcctgagctcgcccgtcacaaagagcttcaacaggggagagtgt

SEQ ID NO: 145 - protein, 215 aa, Artificial Sequence
  source: /note="Description of Artificial Sequence: Synthetic polypeptide"
DIQMTQSPSSLSASVGDRVTITCQASQSISSDYLHWYQQKPGKAPKLLIYRTSNLETGVPSRFSGSGSGTDFTFTISSLQPEDIATYYCQQGTSLPRAFGQGTKLEIKRTVAAPSVFIFPPSDEQLKSGTASVVCLLNNFYPREAKVQWKVDNALQSGNSQESVTEQDSKDSTYSLSSTLTLSKADYEKHKVYACEVTHQGLSSPVTKSFNRGEC

SEQ ID NO: 146 - DNA, 1332 bp, Artificial Sequence
  source: /note="Description of Artificial Sequence: Synthetic polynucleotide"
gaagtgcagctggtggaaagcggcggaggcctggtgcagccaggcggcagcctgagactgagctgcgccgccagcggcttcaccttcagcgactactacatgagctgggtgcgccaggccccaggcaagggcctggagtgggtggcctacatcagcagcggcggcggcagcagctactacccagacctggtgaagggccgcttcaccatcagccgcgacaacgccaagaacagcctgtacctgcagatgcagagcctgcgcgccgaggacaccgccgtgtactactgcgcccgcctgccacactacttcgccatggactactggggccagggcaccctggtgaccgtgagcagcgcctccacaaagggcccttccgtgttccccctggccccttgctcccggtccacctccgagtctaccgccgctctgggctgcctggtcaaggactacttccccgagcccgtgaccgtgtcctggaactctggcgccctgacctccggcgtgcacaccttccctgctgtgctgcagtcctccggcctgtactccctgtcctccgtcgtgaccgtgccctcctctagcctgggcaccaagacctacacctgtaacgtggaccacaagccctccaacaccaaggtggacaagcgggtggaatctaagtacggccctccctgccccccctgccctgcccctgaatttctgggcggaccctccgtgttcctgttccccccaaagcccaaggacaccctgatgatctcccggacccccgaagtgacctgcgtggtggtggacgtgtcccaggaagatcccgaggtccagtttaattggtacgtggacggcgtggaagtgcacaacgccaagaccaagcccagagaggaacagttcaactccacctaccgggtggtgtccgtgctgaccgtgctgcaccaggactggctgaacggcaaagagtacaagtgcaaggtgtccaacaagggcctgccctccagcatcgaaaagaccatctccaaggccaagggccagccccgcgagccccaggtgtacaccctgcctccaagccaggaagagatgaccaagaaccaggtgtccctgacctgtctggtcaagggcttctacccctccgatatcgccgtggaatgggagtccaacggccagcccgagaacaactacaagaccaccccccctgtgctggactccgacggctccttcttcctgtactctcggctgaccgtggacaagtcccggtggcaggaaggcaacgtcttctcctgctccgtgatgcacgaggccctgcacaaccactacacccagaagtccctgtccctgagcctgggc

SEQ ID NO: 147 - protein, 444 aa, Artificial Sequence
  source: /note="Description of Artificial Sequence: Synthetic polypeptide"
EVQLVESGGGLVQPGGSLRLSCAASGFTFSDYYMSWVRQAPGKGLEWVAYISSGGGSSYYPDLVKGRFTISRDNAKNSLYLQMQSLRAEDTAVYYCARLPHYFAMDYWGQGTLVTVSSASTKGPSVFPLAPCSRSTSESTAALGCLVKDYFPEPVTVSWNSGALTSGVHTFPAVLQSSGLYSLSSVVTVPSSSLGTKTYTCNVDHKPSNTKVDKRVESKYGPPCPPCPAPEFLGGPSVFLFPPKPKDTLMISRTPEVTCVVVDVSQEDPEVQFNWYVDGVEVHNAKTKPREEQFNSTYRVVSVLTVLHQDWLNGKEYKCKVSNKGLPSSIEKTISKAKGQPREPQVYTLPPSQEEMTKNQVSLTCLVKGFYPSDIAVEWESNGQPENNYKTTPPVLDSDGSFFLYSRLTVDKSRWQEGNVFSCSVMHEALHNHYTQKSLSLSLG

SEQ ID NO: 148 - DNA, 1332 bp, Artificial Sequence
  source: /note="Description of Artificial Sequence: Synthetic polynucleotide"
gaggtgcagctggtggagagcggcggcggcctggtgcagccaggtggtagcctgcgcctgagctgcgccgccagcggcttcaccttcagcgactactacatgagctgggtgcgccaggctccaggcaagggtctggaatgggtggcctacatcagcagcggcggcggcagcagctactacccagacgccgtgaagggccgcttcaccatcagccgcgacaacgccaagcagagcctgtacctgcagatgcagagcctgcgcgccgaggacaccgccgtgtactactgcgcccgcctgccacactacttcgccatggactactggggccagggcaccctggtgaccgtgagcagcgcctccacaaagggcccttccgtgttccccctggccccttgctcccggtccacctccgagtctaccgccgctctgggctgcctggtcaaggactacttccccgagcccgtgaccgtgtcctggaactctggcgccctgacctccggcgtgcacaccttccctgctgtgctgcagtcctccggcctgtactccctgtcctccgtcgtgaccgtgccctcctctagcctgggcaccaagacctacacctgtaacgtggaccacaagccctccaacaccaaggtggacaagcgggtggaatctaagtacggccctccctgccccccctgccctgcccctgaatttctgggcggaccctccgtgttcctgttccccccaaagcccaaggacaccctgatgatctcccggacccccgaagtgacctgcgtggtggtggacgtgtcccaggaagatcccgaggtccagtttaattggtacgtggacggcgtggaagtgcacaacgccaagaccaagcccagagaggaacagttcaactccacctaccgggtggtgtccgtgctgaccgtgctgcaccaggactggctgaacggcaaagagtacaagtgcaaggtgtccaacaagggcctgccctccagcatcgaaaagaccatctccaaggccaagggccagccccgcgagccccaggtgtacaccctgcctccaagccaggaagagatgaccaagaaccaggtgtccctgacctgtctggtcaagggcttctacccctccgatatcgccgtggaatgggagtccaacggccagcccgagaacaactacaagaccaccccccctgtgctggactccgacggctccttcttcctgtactctcggctgaccgtggacaagtcccggtggcaggaaggcaacgtcttctcctgctccgtgatgcacgaggccctgcacaaccactacacccagaagtccctgtccctgagcctgggc

SEQ ID NO: 149 - protein, 444 aa, Artificial Sequence
  source: /note="Description of Artificial Sequence: Synthetic polypeptide"
EVQLVESGGGLVQPGGSLRLSCAASGFTFSDYYMSWVRQAPGKGLEWVAYISSGGGSSYYPDAVKGRFTISRDNAKQSLYLQMQSLRAEDTAVYYCARLPHYFAMDYWGQGTLVTVSSASTKGPSVFPLAPCSRSTSESTAALGCLVKDYFPEPVTVSWNSGALTSGVHTFPAVLQSSGLYSLSSVVTVPSSSLGTKTYTCNVDHKPSNTKVDKRVESKYGPPCPPCPAPEFLGGPSVFLFPPKPKDTLMISRTPEVTCVVVDVSQEDPEVQFNWYVDGVEVHNAKTKPREEQFNSTYRVVSVLTVLHQDWLNGKEYKCKVSNKGLPSSIEKTISKAKGQPREPQVYTLPPSQEEMTKNQVSLTCLVKGFYPSDIAVEWESNGQPENNYKTTPPVLDSDGSFFLYSRLTVDKSRWQEGNVFSCSVMHEALHNHYTQKSLSLSLG

SEQ ID NO: 150 - DNA, 645 bp, Artificial Sequence
  source: /note="Description of Artificial Sequence: Synthetic polynucleotide"
gacatccagatgacccagagcccaagcagcctgagcgccagcgtgggcgaccgcgtgaccatcacctgccaggccagccagagcatcagcagcgactacctgcactggtaccagcagaagccaggcaaggccccaaagctgctgatctaccgcaccagcaacctggagagcggcgtgccaagccgcttcagcggcagcggcagcggcaccgacttcaccttcaccatcagcagcctgcagccagaggacatcgccacctactactgccagcagggcaccagcctgccacgcgccttcggccagggcaccaagctggagatcaagcgtactgtggctgcaccatctgtcttcatcttcccgccatctgatgagcaattgaaatctggaactgcctctgttgtgtgcctgctgaataacttctatcccagagaggccaaagtacagtggaaggtggataacgccctccaatcgggtaactcccaggagagtgtcacagagcaggacagcaaggacagcacctacagcctcagcagcaccctgacgctgagcaaagcagactacgagaaacacaaagtctacgcctgcgaagtcacccatcagggcctgagctcgcccgtcacaaagagcttcaacaggggagagtgt

SEQ ID NO: 151 - protein, 215 aa, Artificial Sequence
  source: /note="Description of Artificial Sequence: Synthetic polypeptide"
DIQMTQSPSSLSASVGDRVTITCQASQSISSDYLHWYQQKPGKAPKLLIYRTSNLESGVPSRFSGSGSGTDFTFTISSLQPEDIATYYCQQGTSLPRAFGQGTKLEIKRTVAAPSVFIFPPSDEQLKSGTASVVCLLNNFYPREAKVQWKVDNALQSGNSQESVTEQDSKDSTYSLSSTLTLSKADYEKHKVYACEVTHQGLSSPVTKSFNRGEC

SEQ ID NO: 152 - DNA, 1332 bp, Artificial Sequence
  source: /note="Description of Artificial Sequence: Synthetic polynucleotide"
gaagtgcagctggtggaaagcggtggtggcctggtgcagccaggcggctccctgcgcctgagctgcgccgcaagcggtttcacctttagcgactactatatgtcctgggtgcgtcaggcgccaggtaaaggtctggaatgggtggcctacatcagctccgggggcggtagcagctactatccggacctggtgaaagggcgctttactatctcccgggataatgcaaaacagagcctgtacctgcagatgaacagcctgcgggcggaagataccgccgtgtattactgtgcgcgtctgccgcattatttcgccatggattactggggccaggggaccctggtgaccgtgagcagcgcctccacaaagggcccttccgtgttccccctggccccttgctcccggtccacctccgagtctaccgccgctctgggctgcctggtcaaggactacttccccgagcccgtgaccgtgtcctggaactctggcgccctgacctccggcgtgcacaccttccctgctgtgctgcagtcctccggcctgtactccctgtcctccgtcgtgaccgtgccctcctctagcctgggcaccaagacctacacctgtaacgtggaccacaagccctccaacaccaaggtggacaagcgggtggaatctaagtacggccctccctgccccccctgccctgcccctgaatttctgggcggaccctccgtgttcctgttccccccaaagcccaaggacaccctgatgatctcccggacccccgaagtgacctgcgtggtggtggacgtgtcccaggaagatcccgaggtccagtttaattggtacgtggacggcgtggaagtgcacaacgccaagaccaagcccagagaggaacagttcaactccacctaccgggtggtgtccgtgctgaccgtgctgcaccaggactggctgaacggcaaagagtacaagtgcaaggtgtccaacaagggcctgccctccagcatcgaaaagaccatctccaaggccaagggccagccccgcgagccccaggtgtacaccctgcctccaagccaggaagagatgaccaagaaccaggtgtccctgacctgtctggtcaagggcttctacccctccgatatcgccgtggaatgggagtccaacggccagcccgagaacaactacaagaccaccccccctgtgctggactccgacggctccttcttcctgtactctcggctgaccgtggacaagtcccggtggcaggaaggcaacgtcttctcctgctccgtgatgcacgaggccctgcacaaccactacacccagaagtccctgtccctgagcctgggc

SEQ ID NO: 153 - protein, 444 aa, Artificial Sequence
  source: /note="Description of Artificial Sequence: Synthetic polypeptide"
EVQLVESGGGLVQPGGSLRLSCAASGFTFSDYYMSWVRQAPGKGLEWVAYISSGGGSSYYPDLVKGRFTISRDNAKQSLYLQMNSLRAEDTAVYYCARLPHYFAMDYWGQGTLVTVSSASTKGPSVFPLAPCSRSTSESTAALGCLVKDYFPEPVTVSWNSGALTSGVHTFPAVLQSSGLYSLSSVVTVPSSSLGTKTYTCNVDHKPSNTKVDKRVESKYGPPCPPCPAPEFLGGPSVFLFPPKPKDTLMISRTPEVTCVVVDVSQEDPEVQFNWYVDGVEVHNAKTKPREEQFNSTYRVVSVLTVLHQDWLNGKEYKCKVSNKGLPSSIEKTISKAKGQPREPQVYTLPPSQEEMTKNQVSLTCLVKGFYPSDIAVEWESNGQPENNYKTTPPVLDSDGSFFLYSRLTVDKSRWQEGNVFSCSVMHEALHNHYTQKSLSLSLG

SEQ ID NO: 154 - DNA, 1332 bp, Artificial Sequence
  source: /note="Description of Artificial Sequence: Synthetic polynucleotide"
gaggtgcagctggtggagagcggcggcggcctggtgcagccaggtggtagcctgcgcctgagctgcgccgccagcggcttcaccttcagcgactactacatgagctgggtgcgccaggctccaggcaagggtctggaatgggtggcctacatcagcagcggcggcggcagcagctactacccagacctggtgaagggccgcttcaccatcagccgcgacaacgccaagcagagcctgtacctgcagatgcagagcctgcgcgccgaggacaccgccgtgtactactgcgcccgcctgccacactacttcgccatggactactggggccagggcaccctggtgaccgtgagcagcgcctccacaaagggcccttccgtgttccccctggccccttgctcccggtccacctccgagtctaccgccgctctgggctgcctggtcaaggactacttccccgagcccgtgaccgtgtcctggaactctggcgccctgacctccggcgtgcacaccttccctgctgtgctgcagtcctccggcctgtactccctgtcctccgtcgtgaccgtgccctcctctagcctgggcaccaagacctacacctgtaacgtggaccacaagccctccaacaccaaggtggacaagcgggtggaatctaagtacggccctccctgccccccctgccctgcccctgaatttctgggcggaccctccgtgttcctgttccccccaaagcccaaggacaccctgatgatctcccggacccccgaagtgacctgcgtggtggtggacgtgtcccaggaagatcccgaggtccagtttaattggtacgtggacggcgtggaagtgcacaacgccaagaccaagcccagagaggaacagttcaactccacctaccgggtggtgtccgtgctgaccgtgctgcaccaggactggctgaacggcaaagagtacaagtgcaaggtgtccaacaagggcctgccctccagcatcgaaaagaccatctccaaggccaagggccagccccgcgagccccaggtgtacaccctgcctccaagccaggaagagatgaccaagaaccaggtgtccctgacctgtctggtcaagggcttctacccctccgatatcgccgtggaatgggagtccaacggccagcccgagaacaactacaagaccaccccccctgtgctggactccgacggctccttcttcctgtactctcggctgaccgtggacaagtcccggtggcaggaaggcaacgtcttctcctgctccgtgatgcacgaggccctgcacaaccactacacccagaagtccctgtccctgagcctgggc

SEQ ID NO: 155 - protein, 444 aa, Artificial Sequence
  source: /note="Description of Artificial Sequence: Synthetic polypeptide"
EVQLVESGGGLVQPGGSLRLSCAASGFTFSDYYMSWVRQAPGKGLEWVAYISSGGGSSYYPDLVKGRFTISRDNAKQSLYLQMQSLRAEDTAVYYCARLPHYFAMDYWGQGTLVTVSSASTKGPSVFPLAPCSRSTSESTAALGCLVKDYFPEPVTVSWNSGALTSGVHTFPAVLQSSGLYSLSSVVTVPSSSLGTKTYTCNVDHKPSNTKVDKRVESKYGPPCPPCPAPEFLGGPSVFLFPPKPKDTLMISRTPEVTCVVVDVSQEDPEVQFNWYVDGVEVHNAKTKPREEQFNSTYRVVSVLTVLHQDWLNGKEYKCKVSNKGLPSSIEKTISKAKGQPREPQVYTLPPSQEEMTKNQVSLTCLVKGFYPSDIAVEWESNGQPENNYKTTPPVLDSDGSFFLYSRLTVDKSRWQEGNVFSCSVMHEALHNHYTQKSLSLSLG

SEQ ID NO: 156 - DNA, 645 bp, Artificial Sequence
  source: /note="Description of Artificial Sequence: Synthetic polynucleotide"
gagatcgtgctgacacagagccctaccacaatggccgcctctccaggcgagaagatcaccatcacatgtagcgccagcagcagcatcagcagcgactacctgcactggtatcagcagaagcctggcttcagccccgagctgctgatctacagaacaagcaatctggccagcggcgtgccagccagattttctggttctggcagcggcaccagctacagcctgacaatcggatccatggaagccgaggacgtggccacctattactgtcagcagggcacaagcctgcctagagcctttggcggaggcaccaagctggaaatcaagcgtactgtggctgcaccatctgtcttcatcttcccgccatctgatgagcaattgaaatctggaactgcctctgttgtgtgcctgctgaataacttctatcccagagaggccaaagtacagtggaaggtggataacgccctccaatcgggtaactcccaggagagtgtcacagagcaggacagcaaggacagcacctacagcctcagcagcaccctgacgctgagcaaagcagactacgagaaacacaaagtctacgcctgcgaagtcacccatcagggcctgagctcgcccgtcacaaagagcttcaacaggggagagtgt

SEQ ID NO: 157 - protein, 215 aa, Artificial Sequence
  source: /note="Description of Artificial Sequence: Synthetic polypeptide"
EIVLTQSPTTMAASPGEKITITCSASSSISSDYLHWYQQKPGFSPELLIYRTSNLASGVPARFSGSGSGTSYSLTIGSMEAEDVATYYCQQGTSLPRAFGGGTKLEIKRTVAAPSVFIFPPSDEQLKSGTASVVCLLNNFYPREAKVQWKVDNALQSGNSQESVTEQDSKDSTYSLSSTLTLSKADYEKHKVYACEVTHQGLSSPVTKSFNRGEC

SEQ ID NO: 158 - DNA, 1341 bp, Artificial Sequence
  source: /note="Description of Artificial Sequence: Synthetic polynucleotide"
gaagtgcagctggtggaatctggcggaggacttgttcaacctggcggcagcctgaaactgtcttgtgccgccagcggcttcaccttcagcgactactacatgagctgggtccgacagacccctgagaagagactggaatgggtcgcctacatcagctctggcggcggaagcagctactaccctgatagcgtgaagggcagattcaccatcagccgggacaacaccaagaacaccctgtacctgcagatgtccagcctgaagtctgaggacaccgccgtgtactactgtgccagactgcctcactacttcgccatggattattggggccagggcaccagcgtgaccgtttcttctgcctccaccaagggcccatcggtcttcccgctagcaccctcctccaagagcacctctgggggcacagcggccctgggctgcctggtcaaggactacttccccgaaccggtgacggtgtcgtggaactcaggcgccctgaccagcggcgtgcacaccttcccggctgtcctacagtcctcaggactctactccctcagcagcgtggtgaccgtgccctccagcagcttgggcacccagacctacatctgcaacgtgaatcacaagcccagcaacaccaaggtggacaagcgcgttgagcccaaatcttgtgacaaaactcacacatgcccaccgtgcccagcacctgaactactagggggaccgtcagtcttcctcttccccccaaaacccaaggacaccctcatgatctcccggacccctgaggtcacatgcgtggtggtggacgtgagccacgaagaccctgaggtcaagttcaactggtacgtggacggcgtggaggtgcataatgccaagacaaagccgcgggaggagcagtacaacagcacgtaccgtgtggtcagcgtcctcaccgtcctgcaccaggactggctgaatggcaaggagtacaagtgcaaggtctccaacaaagccctcccagcccccatcgagaaaaccatctccaaagccaaagggcagccccgagaaccacaggtgtacaccctgcccccatcccgcgaggagatgaccaagaaccaggtaagtttgacctgcctggtcaaaggcttctatcccagcgacatcgccgtggagtgggagagcaatgggcagccggagaacaactacaagaccacgcctcccgtgctggactccgacggctccttcttcctctatagcaagctcaccgtggacaagagcaggtggcagcaggggaacgtcttctcatgctccgtgatgcatgaggctctgcacaaccactacacgcagaagagcctctccctgtctccgggt

SEQ ID NO: 159 - protein, 447 aa, Artificial Sequence
  source: /note="Description of Artificial Sequence: Synthetic polypeptide"
EVQLVESGGGLVQPGGSLKLSCAASGFTFSDYYMSWVRQTPEKRLEWVAYISSGGGSSYYPDSVKGRFTISRDNTKNTLYLQMSSLKSEDTAVYYCARLPHYFAMDYWGQGTSVTVSSASTKGPSVFPLAPSSKSTSGGTAALGCLVKDYFPEPVTVSWNSGALTSGVHTFPAVLQSSGLYSLSSVVTVPSSSLGTQTYICNVNHKPSNTKVDKRVEPKSCDKTHTCPPCPAPELLGGPSVFLFPPKPKDTLMISRTPEVTCVVVDVSHEDPEVKFNWYVDGVEVHNAKTKPREEQYNSTYRVVSVLTVLHQDWLNGKEYKCKVSNKALPAPIEKTISKAKGQPREPQVYTLPPSREEMTKNQVSLTCLVKGFYPSDIAVEWESNGQPENNYKTTPPVLDSDGSFFLYSKLTVDKSRWQQGNVFSCSVMHEALHNHYTQKSLSLSPG

SEQ ID NO: 160 - DNA, 1341 bp, Artificial Sequence
  source: /note="Description of Artificial Sequence: Synthetic polynucleotide"
gaagtgcagctggtggaatctggcggaggacttgttcaacctggcggcagcctgaaactgtcttgtgccgccagcggcttcaccttcagcgactactacatgagctgggtccgacagacccctgagaagagactggaatgggtcgcctacatcagctctggcggcggaagcagctactaccctgatagcgtgaagggcagattcaccatcagccgggacaacaccaagaacaccctgtacctgcagatgtccagcctgaagtctgaggacaccgccgtgtactactgtgccagactgcctcactacttcgccatggattgttggggccagggcacatctgtgaccgttagttctgcctccaccaagggcccatcggtcttcccgctagcaccctcctccaagagcacctctgggggcacagcggccctgggctgcctggtcaaggactacttccccgaaccggtgacggtgtcgtggaactcaggcgccctgaccagcggcgtgcacaccttcccggctgtcctacagtcctcaggactctactccctcagcagcgtggtgaccgtgccctccagcagcttgggcacccagacctacatctgcaacgtgaatcacaagcccagcaacaccaaggtggacaagcgcgttgagcccaaatcttgtgacaaaactcacacatgcccaccgtgcccagcacctgaagccgctgggggaccgtcagtcttcctcttccccccaaaacccaaggacaccctcatgatctcccggacccctgaggtcacatgcgtggtggtggacgtgagccacgaagaccctgaggtcaagttcaactggtacgtggacggcgtggaggtgcataatgccaagacaaagccgcgggaggagcagtacaacagcacgtaccgtgtggtcagcgtcctcaccgtcctgcaccaggactggctgaatggcaaggagtacaagtgcaaggtctccaacaaagccctcccagcccccatcgagaaaaccatctccaaagccaaagggcagccccgagaaccacaggtgtacaccctgcccccatcccgcgaggagatgaccaagaaccaggtaagtttgacctgcctggtcaaaggcttctatcccagcgacatcgccgtggagtgggagagcaatgggcagccggagaacaactacaagaccacgcctcccgtgctggactccgacggctccttcttcctctatagcaagctcaccgtggacaagagcaggtggcagcaggggaacgtcttctcatgctccgtgatgcatgaggctctgcacaaccactacacgcagaagagcctctccctgtctccgggt

SEQ ID NO: 161 - protein, 447 aa, Artificial Sequence
  source: /note="Description of Artificial Sequence: Synthetic polypeptide"
EVQLVESGGGLVQPGGSLKLSCAASGFTFSDYYMSWVRQTPEKRLEWVAYISSGGGSSYYPDSVKGRFTISRDNTKNTLYLQMSSLKSEDTAVYYCARLPHYFAMDCWGQGTSVTVSSASTKGPSVFPLAPSSKSTSGGTAALGCLVKDYFPEPVTVSWNSGALTSGVHTFPAVLQSSGLYSLSSVVTVPSSSLGTQTYICNVNHKPSNTKVDKRVEPKSCDKTHTCPPCPAPEAAGGPSVFLFPPKPKDTLMISRTPEVTCVVVDVSHEDPEVKFNWYVDGVEVHNAKTKPREEQYNSTYRVVSVLTVLHQDWLNGKEYKCKVSNKALPAPIEKTISKAKGQPREPQVYTLPPSREEMTKNQVSLTCLVKGFYPSDIAVEWESNGQPENNYKTTPPVLDSDGSFFLYSKLTVDKSRWQQGNVFSCSVMHEALHNHYTQKSLSLSPG

SEQ ID NO: 162 - DNA, 1332 bp, Artificial Sequence
  source: /note="Description of Artificial Sequence: Synthetic polynucleotide"
gaagtgcagctggtggaatctggcggaggacttgttcaacctggcggcagcctgaaactgtcttgtgccgccagcggcttcaccttcagcgactactacatgagctgggtccgacagacccctgagaagagactggaatgggtcgcctacatcagctctggcggcggaagcagctactaccctgatagcgtgaagggcagattcaccatcagccgggacaacaccaagaacaccctgtacctgcagatgtccagcctgaagtctgaggacaccgccgtgtactactgtgccagactgcctcactacttcgccatggattattggggccagggcaccagcgtgaccgtttcttctgcctccacaaagggcccttccgtgttccccctggccccttgctcccggtccacctccgagtctaccgccgctctgggctgcctggtcaaggactacttccccgagcccgtgaccgtgtcctggaactctggcgccctgacctccggcgtgcacaccttccctgctgtgctgcagtcctccggcctgtactccctgtcctccgtcgtgaccgtgccctcctctagcctgggcaccaagacctacacctgtaacgtggaccacaagccctccaacaccaaggtggacaagcgggtggaatctaagtacggccctccctgccccccctgccctgcccctgaatttctgggcggaccctccgtgttcctgttccccccaaagcccaaggacaccctgatgatctcccggacccccgaagtgacctgcgtggtggtggacgtgtcccaggaagatcccgaggtccagtttaattggtacgtggacggcgtggaagtgcacaacgccaagaccaagcccagagaggaacagttcaactccacctaccgggtggtgtccgtgctgaccgtgctgcaccaggactggctgaacggcaaagagtacaagtgcaaggtgtccaacaagggcctgccctccagcatcgaaaagaccatctccaaggccaagggccagccccgcgagccccaggtgtacaccctgcctccaagccaggaagagatgaccaagaaccaggtgtccctgacctgtctggtcaagggcttctacccctccgatatcgccgtggaatgggagtccaacggccagcccgagaacaactacaagaccaccccccctgtgctggactccgacggctccttcttcctgtactctcggctgaccgtggacaagtcccggtggcaggaaggcaacgtcttctcctgctccgtgatgcacgaggccctgcacaaccactacacccagaagtccctgtccctgagcctgggc

SEQ ID NO: 163 - protein, 444 aa, Artificial Sequence
  source: /note="Description of Artificial Sequence: Synthetic polypeptide"
EVQLVESGGGLVQPGGSLKLSCAASGFTFSDYYMSWVRQTPEKRLEWVAYISSGGGSSYYPDSVKGRFTISRDNTKNTLYLQMSSLKSEDTAVYYCARLPHYFAMDYWGQGTSVTVSSASTKGPSVFPLAPCSRSTSESTAALGCLVKDYFPEPVTVSWNSGALTSGVHTFPAVLQSSGLYSLSSVVTVPSSSLGTKTYTCNVDHKPSNTKVDKRVESKYGPPCPPCPAPEFLGGPSVFLFPPKPKDTLMISRTPEVTCVVVDVSQEDPEVQFNWYVDGVEVHNAKTKPREEQFNSTYRVVSVLTVLHQDWLNGKEYKCKVSNKGLPSSIEKTISKAKGQPREPQVYTLPPSQEEMTKNQVSLTCLVKGFYPSDIAVEWESNGQPENNYKTTPPVLDSDGSFFLYSRLTVDKSRWQEGNVFSCSVMHEALHNHYTQKSLSLSLG

SEQ ID NO: 164 - protein, 12 aa, Artificial Sequence
  source: /note="Description of Artificial Sequence: Synthetic peptide"
SASQSISSDYLH

SEQ ID NO: 165 - protein, 12 aa, Artificial Sequence
  source: /note="Description of Artificial Sequence: Synthetic peptide"
QASQSISSDYLH

SEQ ID NO: 166 - protein, 7 aa, Artificial Sequence
  source: /note="Description of Artificial Sequence: Synthetic peptide"
RTSNLET

SEQ ID NO: 167 - protein, 7 aa, Artificial Sequence
  source: /note="Description of Artificial Sequence: Synthetic peptide"
RTSNLES